European Patent Application EP 4 124 621 A1, published February 1, 2023. Title: carrier peptide fragment for nucleolar localization and use thereof. Applicant: TOAGOSEI CO., LTD. The sequence listing filed with the application follows.

SEQUENCE LISTING (6 sequences)

SEQ ID NO: 1 - protein, 13 aa, synthetic construct
  REGION 1..13: note = synthetic peptide
KKRTLRKKKRKKR

SEQ ID NO: 2 - protein, 13 aa, synthetic construct
  REGION 1..13: note = synthetic peptide
KKRTLRKRRRKKR

SEQ ID NO: 3 - protein, 13 aa, synthetic construct
  REGION 1..13: note = synthetic peptide
KKRTLRKRKRKKR

SEQ ID NO: 4 - protein, 13 aa, synthetic construct
  REGION 1..13: note = synthetic peptide
KKRTLRKKRRKKR

SEQ ID NO: 5 - protein, 13 aa, synthetic construct
  REGION 1..13: note = synthetic peptide
KKRTLRKNDRKKR

SEQ ID NO: 6 - protein, 8 aa, synthetic construct
  REGION 1..8: note = synthetic peptide
RRRRRRRR